European Patent Specification EP 4 587 833 B1, published February 25, 2026. Title: IMMUNOASSAY ZUM NACHWEISEN BIOLOGISCH AKTIVER PROTEINE. Applicant: Phaeosynt GmbH. Application EP PCT/EP2023/075545, filed September 15, 2023. The sequence listing filed with the application follows.

SEQUENCE LISTING (5 sequences)

SEQ ID NO: 1 - DNA, 864 bp, synthetic construct
  source 1..864: mol_type = other DNA
catacagtgaatgtaactttcgaattgacagtattagtagtcgtattgacagtgaggcacgcccctcaatgtgcgaggtggaaaatataccagcatgacaatgaatcttggagattcttttgctgtcatcaagattcaccgccaaatcttcaggaacctatcacgtccacaggcgatgttaattcttgagtcgtcaaaacaaagtcctgtcctacctgtagaagttgacagcgagcaattgtatgcaaacttctgactttgttataataacattaaaggtaattaagtatcttcaattaggcattttgtcactgtcagtccgttccgacaatataggtagatttggaatgaatcttttctatgctcatacagtgaatgtaactttcgaattgacagtattagtagtcgtattgacagtgaggcacgcccctcaatgtgcgaggtggaaaatataccagcatgacaatgaatcttggagattcttttgctgtcatcaagattcaccgccaaatcttcaggaacctatcacgtccacaggcgatgttaattcttgagtcgtcaaaacaaagtcctgtcctacctgtagaagttgacagcgagcaattgtatgcaaacttctgactttgttataataacattaaaggtaattaagtatcttcaattaggcattttgtcactgtcagtccgttccgacaatataggtagatttggaatgaatcttttctatgctgctgcgaatcttgtacacctttgaggccgtagattctgtccgacgaagcgataattattgcaaaatacatggactcattattttgattcgatttctttttggtatccgactcgaaaagatccatcacggcgagc

SEQ ID NO: 2 - protein, 12 aa, synthetic construct
VIKEPCCCPKCP

SEQ ID NO: 3 - protein, 10 aa, synthetic construct
EQKLISEEDL

SEQ ID NO: 4 - protein, 8 aa, synthetic construct
WSHPQFEK

SEQ ID NO: 5 - protein, 8 aa, synthetic construct
DYKDDDDK